European Patent Specification EP 3 982 749 B1, published July 15, 2026. Title: COMPOSITIONS AND METHODS FOR GROWING THE POPULATION OF MICROORGANISMS IN A GUT OF MONOGASTRIC ANIMALS. Applicant: DANSTAR FERMENT AG. Application tba. The sequence listing filed with the application follows.

SEQUENCE LISTING (4 sequences)

SEQ ID NO: 1 - DNA, 42 bp, Artificial Sequence
  V3V4-343F primer
  misc_feature (33)..(33): A or G
ctttccctacacgacgctcttccgatctacggraggcagcag

SEQ ID NO: 2 - DNA, 47 bp, Artificial Sequence
  V3V4-783R primer
ggagttcagacgtgtgctcttccgatcttaccagggtatctaatcct

SEQ ID NO: 3 - DNA, 46 bp, Artificial Sequence
  V4V5-515F primer
  misc_feature (32)..(32): C or T
  misc_feature (37)..(37): A or C
ctttccctacacgacgctcttccgatctgtgycagcmgccgcggta

SEQ ID NO: 4 - DNA, 48 bp, Artificial Sequence
  V4V5-928R primer
  misc_feature (34)..(34): C or T
  misc_feature (41)..(41): A or C
  misc_feature (45)..(45): A or G
ggagttcagacgtgtgctcttccgatctccccgycaattcmtttragt